European Patent Specification EP 3 934 712 B1, published February 18, 2026. Title: BLOOD TREATMENT DEVICE COMPRISING ALKALINE PHOSPHATASE. Applicant: Gambro Lundia AB. The sequence listing filed with the application follows.

SEQUENCE LISTING (6 sequences)

SEQ ID NO: 1 - protein, 533 aa, Bos taurus
MQGACVLLLLGLHLQLSLGLVPVEEEDPAFWNRQAAQALDVAKKLQPIQTAAKNVILFLGDGMGVPTVTATRILKGQMNGKLGPETPLAMDQFPYVALSKTYNVDRQVPDSAGTATAYLCGVKGNYRTIGVSAAARYNQCKTTRGNEVTSVMNRAKKAGKSVGVVTTTRVQHASPAGAYAHTVNRNWYSDADLPADAQMNGCQDIAAQLVNNMDIDVILGGGRKYMFPVGTPDPEYPDDASVNGVRKRKQNLVQAWQAKHQGAQYVWNRTALLQAADDSSVTHLMGLFEPADMKYNVQQDHTKDPTLQEMTEVALRVVSRNPRGFYLFVEGGRIDHGHHDDKAYMALTEAGMFDNAIAKANELTSELDTLILVTADHSHVFSFGGYTLRGTSIFGLAPSKALDSKSYTSILYGNGPGYALGGGSRPDVNDSTSEDPSYQQQAAVPQASETHGGEDVAVFARGPQAHLVHGVEEETFVAHIMAFAGCVEPYTDCNLPAPTTATSIPDAAHLAASPPPLALLAGAMLLLLAPTLY

SEQ ID NO: 2 - protein, 532 aa, Homo sapiens [sequence omitted]

SEQ ID NO: 3 - protein, 524 aa, Homo sapiens
MISPFLVLAIGTCLTNSLVPEKEKDPKYWRDQAQETLKYALELQKLNTNVAKNVIMFLGDGMGVSTVTAARILKGQLHHNPGEETRLEMDKFPFVALSKTYNTNAQVPDSAGTATAYLCGVKANEGTVGVSAATERSRCNTTQGNEVTSILRWAKDAGKSVGIVTTTRVNHATPSAAYAHSADRDWYSDNEMPPEALSQGCKDIAYQLMHNIRDIDVIMGGGRKYMYPKNKTDVEYESDEKARGTRLDGLDLVDTWKSFKPRYKHSHFIWNRTELLTLDPHNVDYLLGLFEPGDMQYELNRNNVTDPSLSEMVVVAIQILRKNPKGFFLLVEGGRIDHGHHEGKAKQALHEAVEMDRAIGQAGSLTSSEDTLTVVTADHSHVFTFGGYTPRGNSIFGLAPMLSDTDKKPFTAILYGNGPGYKVVGGERENVSMVDYAHNNYQAQSAVPLRHETHGGEDVAVFSKGPMAHLLHGVHEQNYVPHVMAYAACIGANLGHCAPASSAGSLAAGPLLLALALYPLSVLF

SEQ ID NO: 4 - protein, 528 aa, Homo sapiens
MQGPWVLLLLGLRLQLSLGVIPAEEENPAFWNRQAAEALDAAKKLQPIQKVAKNLILFLGDGLGVPTVTATRILKGQKNGKLGPETPLAMDRFPYLALSKTYNVDRQVPDSAATATAYLCGVKANFQTIGLSAAARFNQCNTTRGNEVISVMNRAKQAGKSVGVVTTTRVQHASPAGTYAHTVNRNWYSDADMPASARQEGCQDIATQLISNMDIDVILGGGRKYMFPMGTPDPEYPADASQNGIRLDGKNLVQEWLAKHQGAWYVWNRTELMQASLDQSVTHLMGLFEPGDTKYEIHRDPTLDPSLMEMTEAALRLLSRNPRGFYLFVEGGRIDHGHHEGVAYQALTEAVMFDDAIERAGQLTSEEDTLTLVTADHSHVFSFGGYTLRGSSIFGLAPSKAQDSKAYTSILYGNGPGYVFNSGVRPDVNESESGSPDYQQQAAVPLSSETHGGEDVAVFARGPQAHLVHGVQEQSFVAHVMAFAACLEPYTACDLAPPACTTDAAHPVAASLPLLAGTLLLLGASAAP

SEQ ID NO: 5 - protein, 509 aa, Homo sapiens
VIPAEEENPAFWNRQAAEALDAAKKLQPIQKVAKNLILFLGDGLGVPTVTATRILKGQKNGKLGPETPLAMDRFPYLALSKTYNVDRQVPDSAATATAYLCGVKANFQTIGLSAAARFNQCNTTRGNEVISVMNRAKQAGKSVGVVTTTRVQHASPAGTYAHTVNRNWYSDADMPASARQEGCQDIATQLISNMDIDVILGGGRKYMFPMGTPDPEYPADASQNGIRLDGKNLVQEWLAKHQGAWYVWNRTELMQASLDQSVTHLMGLFEPGDTKYEIHRDPTLDPSLMEMTEAALRLLSRNPRGFYLFVEGGRIDHGHHEGVAYQALTEAVMFDDAIERAGQLTSEEDTLTLVTADHSHVFSFGGYTLRGSSIFGLAPSKAQDSKAYTSILYGNGPGYVFNSGVRPDVNESESGSPDYQQQAAVPLSSETHGGEDVAVFARGPQAHLVHGVQEQSFVAHVMAFAACLEPYTACDLAPPACTTDAAHPVAASLPLLAGTLLLLGASAAP

SEQ ID NO: 6 - protein, 484 aa, Artificial Sequence
  Recombinant AP
VIPAEEENPAFWNRQAAEALDAAKKLQPIQKVAKNLILFLGDGLGVPTVTATRILKGQKNGKLGPETPLAMDRFPYLALSKTYNVDRQVPDSAATATAYLCGVKANFQTIGLSAAARFNQCNTTRGNEVISVMNRAKQAGKSVGVVTTTRVQHASPAGTYAHTVNRNWYSDADMPASARQEGCQDIATQLISNMDIDVILGGGRKYMFPMGTPDPEYPADASQNGIRLDGKNLVQEWLAKHQGAWYVWNRTELMQASLDQSVTHLMGLFEPGDTKYEIHRDPTLDPSLMEMTEAALRLLSRNPRGFYLFVEGGRIDHGHHEGVAYQALTEAVMFDDAIERAGQLTSEEDTLTLVTADHSHVFSFGGYPLRGSSIFGLAPGKARDRKAYTVLLYGNGPGYVLKDGARPDVTESESGSPEYRQQSAVPLDEETHGGEDVAVFARGPQAHLVHGVQEQSFVAHVMAFAACLEPYTACDLAPPACTTD